European Patent Application EP 4 269 439 A2, published November 1, 2023. Title: REDUCING SYSTEMIC REGULATORY T CELL LEVELS OR ACTIVITY FOR TREATMENT OF DISEASE AND INJURY OF THE CNS. Applicant: Yeda Research and Development Co. Ltd. The sequence listing filed with the application follows.

SEQUENCE LISTING (56 sequences)

SEQ ID NO: 1-32 - skipped (32 entries)

SEQ ID NO: 33 - DNA, 24 bp, synthetic construct
  source 1..24: mol_type = other DNA; note = Synthetic
agcatacaggtcctggcatcttgt

SEQ ID NO: 34 - DNA, 24 bp, synthetic construct
  source 1..24: mol_type = other DNA; note = Synthetic
caaagaccacatgcttgccatcca

SEQ ID NO: 35 - DNA, 24 bp, synthetic construct
  source 1..24: mol_type = other DNA; note = Synthetic
agatcacattcacggtgctggcta

SEQ ID NO: 36 - DNA, 24 bp, synthetic construct
  source 1..24: mol_type = other DNA; note = Synthetic
agctttgggatggtagctggaaga

SEQ ID NO: 37 - DNA, 24 bp, synthetic construct
  source 1..24: mol_type = other DNA; note = Synthetic
tgtgaagggattaacgaggctgga

SEQ ID NO: 38 - DNA, 24 bp, synthetic construct
  source 1..24: mol_type = other DNA; note = Synthetic
ccatgtttcgggcacatttccaca

SEQ ID NO: 39 - DNA, 21 bp, synthetic construct
  source 1..21: mol_type = other DNA; note = Synthetic
aactgcatccatatcgatgac

SEQ ID NO: 40 - DNA, 19 bp, synthetic construct
  source 1..19: mol_type = other DNA; note = Synthetic
gtggcaatgatctcaacac

SEQ ID NO: 41 - DNA, 18 bp, synthetic construct
  source 1..18: mol_type = other DNA; note = Synthetic
catccacgtgttggctca

SEQ ID NO: 42 - DNA, 23 bp, synthetic construct
  source 1..23: mol_type = other DNA; note = Synthetic
gatcatcttgctggtgaatgagt

SEQ ID NO: 43 - DNA, 20 bp, synthetic construct
  source 1..20: mol_type = other DNA; note = Synthetic
gcctcttctcattcctgctt

SEQ ID NO: 44 - DNA, 20 bp, synthetic construct
  source 1..20: mol_type = other DNA; note = Synthetic
ctcctccacttggtggtttg

SEQ ID NO: 45 - DNA, 21 bp, synthetic construct
  source 1..21: mol_type = other DNA; note = Synthetic
ccaaaagatgaagggctgctt

SEQ ID NO: 46 - DNA, 20 bp, synthetic construct
  source 1..20: mol_type = other DNA; note = Synthetic
tgctgctgcgagatttgaag

SEQ ID NO: 47 - DNA, 20 bp, synthetic construct
  source 1..20: mol_type = other DNA; note = Synthetic
gaagttcaacatcaagagca

SEQ ID NO: 48 - DNA, 19 bp, synthetic construct
  source 1..19: mol_type = other DNA; note = Synthetic
catagtccctttggtccag

SEQ ID NO: 49 - DNA, 24 bp, synthetic construct
  source 1..24: mol_type = other DNA; note = Synthetic
tgaattccctgggtgagaagctga

SEQ ID NO: 50 - DNA, 24 bp, synthetic construct
  source 1..24: mol_type = other DNA; note = Synthetic
tggccttgtagacaccttggtctt

SEQ ID NO: 51 - DNA, 24 bp, synthetic construct
  source 1..24: mol_type = other DNA; note = Synthetic
aattgctgccttcgccctctttac

SEQ ID NO: 52 - DNA, 24 bp, synthetic construct
  source 1..24: mol_type = other DNA; note = Synthetic
tgtacaggctgaggactttggtgt

SEQ ID NO: 53 - DNA, 19 bp, synthetic construct
  source 1..19: mol_type = other DNA; note = Synthetic
ccggaccagagaccctttg

SEQ ID NO: 54 - DNA, 23 bp, synthetic construct
  source 1..23: mol_type = other DNA; note = Synthetic
cctgtgggcttgttgaagtaaaa

SEQ ID NO: 55 - DNA, 24 bp, synthetic construct
  source 1..24: mol_type = other DNA; note = Synthetic
gatgctcagcagtcaagtgccttt

SEQ ID NO: 56 - DNA, 24 bp, synthetic construct
  source 1..24: mol_type = other DNA; note = Synthetic
gacatgtttgcggcatccaggtaa